European Patent Specification EP 4 053 145 B1, published June 12, 2024. Title: BICYCLIC PEPTIDE LIGANDS SPECIFIC FOR EphA2. Applicant: BicycleTx Limited. The sequence listing filed with the application follows.

SEQUENCE LISTING (3 sequences)

SEQ ID NO: 1 - protein, 15 aa, Artificial
  Synthetic Peptide
  Xaa (2)..(2): X represents HyP
  Xaa (12)..(12): Xaa represents D-Asp
  Xaa (14)..(14): Xaa represents HArg
CXLVNPLCLHPXWXC

SEQ ID NO: 2 - protein, 20 aa, Artificial
  Synthetic Peptide
  Xaa (1)..(1): Xaa represents Beta-Ala
  Xaa (2)..(2): Xaa represents Sar10
  Xaa (4)..(4): Xaa represents HArg
  Xaa (7)..(7): Xaa represents HyP
  Xaa (17)..(17): Xaa represents D-Asp
  Xaa (19)..(19): Xaa represents HArg
XXAXDCXLVNPLCLHPXWXC

SEQ ID NO: 3 - protein, 7 aa, Artificial
  Synthetic Linker
  Xaa (3)..(3): Xaa represents Cit
  Xaa (5)..(5): Xaa represents hPhe
EPXGXYL